European Patent Application EP 4 141 111 A1, published March 1, 2023. Title: 一种溶瘤病毒疫苗及其与免疫细胞联合治疗肿瘤的药物. Applicant: 上海荣瑞医药科技有限公司. The sequence listing filed with the application follows.

SEQUENCE LISTING (13 sequences)

SEQ ID NO: 1 - DNA, 690 bp, 水疱性口炎病毒印第安纳株(VSV MuddSummer)
atgagttccttaaagaagattctcggtctgaaggggaaaggtaagaaatctaagaaattagggatcgcaccacccccttatgaagaggacactagcatggagtatgctccgagcgctccaattgacaaatcctattttggagttgacgagatggacacctatgatccgaatcaattaagatatgagaaattcttctttacagtgaaaatgacggttagatctaatcgtccgttcagaacatactcagatgtggcagccgctgtatcccattgggatcacatgtacatcggaatggcagggaaacgtcccttctacaaaatcttggcttttttgggttcttctaatctaaaggccactccagcggtattggcagatcaaggtcaaccagagtatcacgctcactgcgaaggcagggcttatttgccacataggatggggaagacccctcccatgctcaatgtaccagagcacttcagaagaccattcaatataggtctttacaagggaacgattgagctcacaatgaccatctacgatgatgagtcactggaagcagctcctatgatctgggatcatttcaattcttccaaattttctgatttcagagagaaggccttaatgtttggcctgattgtcgagaaaaaggcatctggagcgtgggtcctggactctatcggccacttcaaatga

SEQ ID NO: 2 - protein, 229 aa, 水疱性口炎病毒印第安纳株(VSV MuddSummer)
MSSLKKILGLKGKGKKSKKLGIAPPPYEEDTSMEYAPSAPIDKSYFGVDEMDTYDPNQLRYEKFFFTVKMTVRSNRPFRTYSDVAAAVSHWDHMYIGMAGKRPFYKILAFLGSSNLKATPAVLADQGQPEYHAHCEGRAYLPHRMGKTPPMLNVPEHFRRPFNIGLYKGTIELTMTIYDDESLEAAPMIWDHFNSSKFSDFREKALMFGLIVEKKASGAWVLDSISHFK

SEQ ID NO: 3 - DNA, 687 bp, 人工序列（Artificial Sequence）
  基质蛋白M（M51R，ΔL111，V221F，S226R）
atgagttccttaaagaagattctcggtctgaaggggaaaggtaagaaatctaagaaattagggatcgcaccacccccttatgaagaggacactagcatggagtatgctccgagcgctccaattgacaaatcctattttggagttgacgagatggacacctatgatccgaatcaattaagatatgagaaattcttctttacagtgaaaatgacggttagatctaatcgtccgttcagaacatactcagatgtggcagccgctgtatcccattgggatcacatgtacatcggaatggcagggaaacgtcccttctacaaaatcttggctttgggttcttctaatctaaaggccactccagcggtattggcagatcaaggtcaaccagagtatcacgctcactgcgaaggcagggcttatttgccacataggatggggaagacccctcccatgctcaatgtaccagagcacttcagaagaccattcaatataggtctttacaagggaacgattgagctcacaatgaccatctacgatgatgagtcactggaagcagctcctatgatctgggatcatttcaattcttccaaattttctgatttcagagagaaggccttaatgtttggcctgattgtcgagaaaaaggcatctggagcgtgggtcctggactctatcggccacttcaaatga

SEQ ID NO: 4 - protein, 228 aa, 人工序列（Artificial Sequence）
  基质蛋白M（M51R，ΔL111，V221F，S226R）（PRT）
MSSLKKILGLKGKGKKSKKLGIAPPPYEEDTSMEYAPSAPIDKSYFGVDERDTYDPNQLRYEKFFFTVKMTVRSNRPFRTYSDVAAAVSHWDHMYIGMAGKRPFYKILAFGSSNLKATPAVLADQGQPEYHAHCEGRAYLPHRMGKTPPMLNVPEHFRRPFNIGLYKGTIELTMTIYDDESLEAAPMIWDHFNSSKFSDFREKALMFGLIVEKKASGAWFLDSIRHFK

SEQ ID NO: 5 - DNA, 20 bp, 人工序列（Artificial Sequence）
  引物1
aaaaaagtaacagatatcac

SEQ ID NO: 6 - DNA, 24 bp, 人工序列（Artificial Sequence）
  引物2
acatttttccagtttcctttttgg

SEQ ID NO: 7 - protein, 228 aa, 人工序列（Artificial Sequence）
  基质蛋白M（ΔL111）
MSSLKKILGLKGKGKKSKKLGIAPPPYEEDTSMEYAPSAPIDKSYFGVDEMDTYDPNQLRYEKFFFTVKMTVRSNRPFRTYSDVAAAVSHWDHMYIGMAGKRPFYKILAFGSSNLKATPAVLADQGQPEYHAHCEGRAYLPHRMGKTPPMLNVPEHFRRPFNIGLYKGTIELTMTIYDDESLEAAPMIWDHFNSSKFSDFREKALMFGLIVEKKASGAWVLDSISHFK

SEQ ID NO: 8 - protein, 228 aa, 人工序列（Artificial Sequence）
  基质蛋白M（ΔL111，M51R）
MSSLKKILGLKGKGKKSKKLGIAPPPYEEDTSMEYAPSAPIDKSYFGVDERDTYDPNQLRYEKFFFTVKMTVRSNRPFRTYSDVAAAVSHWDHMYIGMAGKRPFYKILAFGSSNLKATPAVLADQGQPEYHAHCEGRAYLPHRMGKTPPMLNVPEHFRRPFNIGLYKGTIELTMTIYDDESLEAAPMIWDHFNSSKFSDFREKALMFGLIVEKKASGAWVLDSISHFK

SEQ ID NO: 9 - protein, 228 aa, 人工序列（Artificial Sequence）
  基质蛋白M（ΔL111，V221F）
MSSLKKILGLKGKGKKSKKLGIAPPPYEEDTSMEYAPSAPIDKSYFGVDEMDTYDPNQLRYEKFFFTVKMTVRSNRPFRTYSDVAAAVSHWDHMYIGMAGKRPFYKILAFGSSNLKATPAVLADQGQPEYHAHCEGRAYLPHRMGKTPPMLNVPEHFRRPFNIGLYKGTIELTMTIYDDESLEAAPMIWDHFNSSKFSDFREKALMFGLIVEKKASGAWFLDSISHFK

SEQ ID NO: 10 - protein, 228 aa, 人工序列（Artificial Sequence）
  基质蛋白M（ΔL111，S226R）
MSSLKKILGLKGKGKKSKKLGIAPPPYEEDTSMEYAPSAPIDKSYFGVDEMDTYDPNQLRYEKFFFTVKMTVRSNRPFRTYSDVAAAVSHWDHMYIGMAGKRPFYKILAFGSSNLKATPAVLADQGQPEYHAHCEGRAYLPHRMGKTPPMLNVPEHFRRPFNIGLYKGTIELTMTIYDDESLEAAPMIWDHFNSSKFSDFREKALMFGLIVEKKASGAWVLDSIRHFK

SEQ ID NO: 11 - protein, 228 aa, 人工序列（Artificial Sequence）
  基质蛋白M（ΔL111，V221F，S226R）
MSSLKKILGLKGKGKKSKKLGIAPPPYEEDTSMEYAPSAPIDKSYFGVDEMDTYDPNQLRYEKFFFTVKMTVRSNRPFRTYSDVAAAVSHWDHMYIGMAGKRPFYKILAFGSSNLKATPAVLADQGQPEYHAHCEGRAYLPHRMGKTPPMLNVPEHFRRPFNIGLYKGTIELTMTIYDDESLEAAPMIWDHFNSSKFSDFREKALMFGLIVEKKASGAWFLDSIRHFK

SEQ ID NO: 12 - DNA, 20 bp, 人工序列（Artificial Sequence）
  引物3
ggaattcatggagaccctct

SEQ ID NO: 13 - DNA, 29 bp, 人工序列（Artificial Sequence）
  引物4
atagtttagcggccgcctagcctctggaa